European Patent Specification EP 3 567 121 B1, published August 30, 2023. Title: WORKFLOW FOR DETECTION OF LIGANDS USING NUCLEIC ACIDS. Applicant: CHEN, SHIAW-MIN SWARTZMAN, ELANA RUFF, DAVID SHANNON, MARK LU, JULIA HENDRICKS, STEPHEN. Application PCT/US2012/021585. The sequence listing filed with the application follows.

SEQUENCE LISTING (84 sequences)

SEQ ID NO: 1 - protein, 9 aa, Artificial Sequence
  Description of Artificial Sequence: Synthetic peptide
ATPKIDGIR

SEQ ID NO: 2 - protein, 8 aa, Artificial Sequence
  Description of Artificial Sequence: Synthetic peptide
EGSDGEIS

SEQ ID NO: 3 - protein, 5 aa, Artificial Sequence
  Description of Artificial Sequence: Synthetic peptide
YWFDY

SEQ ID NO: 4 - protein, 6 aa, Artificial Sequence
  Description of Artificial Sequence: Synthetic peptide
EGVMIR

SEQ ID NO: 5 - protein, 5 aa, Artificial Sequence
  Description of Artificial Sequence: Synthetic peptide
LLKMK

SEQ ID NO: 6 - protein, 9 aa, Artificial Sequence
  Description of Artificial Sequence: Synthetic peptide
CELKLDGLA

SEQ ID NO: 7 - protein, 9 aa, Artificial Sequence
  Description of Artificial Sequence: Synthetic peptide
VEHKVDGLS

SEQ ID NO: 8 - protein, 9 aa, Artificial Sequence
  Description of Artificial Sequence: Synthetic peptide
CEPKLDGLA

SEQ ID NO: 9 - protein, 9 aa, Artificial Sequence
  Description of Artificial Sequence: Synthetic peptide
CELKLDGVA

SEQ ID NO: 10 - protein, 9 aa, Artificial Sequence
  Description of Artificial Sequence: Synthetic peptide
AEIKYDGVR

SEQ ID NO: 11 - protein, 9 aa, Artificial Sequence
  Description of Artificial Sequence: Synthetic peptide
CEYKYDGQR

SEQ ID NO: 12 - protein, 9 aa, Artificial Sequence
  Description of Artificial Sequence: Synthetic peptide
VDYKYDGER

SEQ ID NO: 13 - protein, 9 aa, Artificial Sequence
  Description of Artificial Sequence: Synthetic peptide
FEIKYDGAR

SEQ ID NO: 14 - protein, 9 aa, Artificial Sequence
  Description of Artificial Sequence: Synthetic peptide
FEGKWDGYR

SEQ ID NO: 15 - protein, 9 aa, Artificial Sequence
  Description of Artificial Sequence: Synthetic peptide
AREKIHGTN

SEQ ID NO: 16 - protein, 9 aa, Artificial Sequence
  Description of Artificial Sequence: Synthetic peptide
ACEKVHGTN

SEQ ID NO: 17 - protein, 9 aa, Artificial Sequence
  Description of Artificial Sequence: Synthetic peptide
ILTKEDGSL

SEQ ID NO: 18 - protein, 9 aa, Artificial Sequence
  Description of Artificial Sequence: Synthetic peptide
VEEKVDGYN

SEQ ID NO: 19 - protein, 8 aa, Artificial Sequence
  Description of Artificial Sequence: Synthetic peptide
LEVRGEVF

SEQ ID NO: 20 - protein, 8 aa, Artificial Sequence
  Description of Artificial Sequence: Synthetic peptide
VEVRGECY

SEQ ID NO: 21 - protein, 8 aa, Artificial Sequence
  Description of Artificial Sequence: Synthetic peptide
LEVRGEVY

SEQ ID NO: 22 - protein, 8 aa, Artificial Sequence
  Description of Artificial Sequence: Synthetic peptide
LEARGEAF

SEQ ID NO: 23 - protein, 8 aa, Artificial Sequence
  Description of Artificial Sequence: Synthetic peptide
FMLDGELM

SEQ ID NO: 24 - protein, 8 aa, Artificial Sequence
  Description of Artificial Sequence: Synthetic peptide
EGSDGEIS

SEQ ID NO: 25 - protein, 8 aa, Artificial Sequence
  Description of Artificial Sequence: Synthetic peptide
FILDTEAV

SEQ ID NO: 26 - protein, 8 aa, Artificial Sequence
  Description of Artificial Sequence: Synthetic peptide
FIIEGEIV

SEQ ID NO: 27 - protein, 8 aa, Artificial Sequence
  Description of Artificial Sequence: Synthetic peptide
AIVEGELV

SEQ ID NO: 28 - protein, 8 aa, Artificial Sequence
  Description of Artificial Sequence: Synthetic peptide
VVLDGEAV

SEQ ID NO: 29 - protein, 8 aa, Artificial Sequence
  Description of Artificial Sequence: Synthetic peptide
YQVFGEFA

SEQ ID NO: 30 - protein, 8 aa, Artificial Sequence
  Description of Artificial Sequence: Synthetic peptide
LVLNGELF

SEQ ID NO: 31 - protein, 8 aa, Artificial Sequence
  Description of Artificial Sequence: Synthetic peptide
FTANFEFV

SEQ ID NO: 32 - protein, 8 aa, Artificial Sequence
  Description of Artificial Sequence: Synthetic peptide
LILVGEMA

SEQ ID NO: 33 - protein, 5 aa, Artificial Sequence
  Description of Artificial Sequence: Synthetic peptide
FCYGV

SEQ ID NO: 34 - protein, 5 aa, Artificial Sequence
  Description of Artificial Sequence: Synthetic peptide
FLYTV

SEQ ID NO: 35 - protein, 5 aa, Artificial Sequence
  Description of Artificial Sequence: Synthetic peptide
TFYAL

SEQ ID NO: 36 - protein, 5 aa, Artificial Sequence
  Description of Artificial Sequence: Synthetic peptide
ICHGL

SEQ ID NO: 37 - protein, 5 aa, Artificial Sequence
  Description of Artificial Sequence: Synthetic peptide
NAYGI

SEQ ID NO: 38 - protein, 5 aa, Artificial Sequence
  Description of Artificial Sequence: Synthetic peptide
FVYGL

SEQ ID NO: 39 - protein, 5 aa, Artificial Sequence
  Description of Artificial Sequence: Synthetic peptide
KLYAI

SEQ ID NO: 40 - protein, 5 aa, Artificial Sequence
  Description of Artificial Sequence: Synthetic peptide
YWFDY

SEQ ID NO: 41 - protein, 5 aa, Artificial Sequence
  Description of Artificial Sequence: Synthetic peptide
YAFDI

SEQ ID NO: 42 - protein, 5 aa, Artificial Sequence
  Description of Artificial Sequence: Synthetic peptide
FLFDL

SEQ ID NO: 43 - protein, 5 aa, Artificial Sequence
  Description of Artificial Sequence: Synthetic peptide
NLFDV

SEQ ID NO: 44 - protein, 5 aa, Artificial Sequence
  Description of Artificial Sequence: Synthetic peptide
WAFDL

SEQ ID NO: 45 - protein, 5 aa, Artificial Sequence
  Description of Artificial Sequence: Synthetic peptide
YVFDI

SEQ ID NO: 46 - protein, 5 aa, Artificial Sequence
  Description of Artificial Sequence: Synthetic peptide
FAFDI

SEQ ID NO: 47 - protein, 5 aa, Artificial Sequence
  Description of Artificial Sequence: Synthetic peptide
ILLNA

SEQ ID NO: 48 - protein, 5 aa, Artificial Sequence
  Description of Artificial Sequence: Synthetic peptide
FLFDV

SEQ ID NO: 49 - protein, 6 aa, Artificial Sequence
  Description of Artificial Sequence: Synthetic peptide
DGVVIK

SEQ ID NO: 50 - protein, 6 aa, Artificial Sequence
  Description of Artificial Sequence: Synthetic peptide
DGIVIK

SEQ ID NO: 51 - protein, 6 aa, Artificial Sequence
  Description of Artificial Sequence: Synthetic peptide
DGVVVK

SEQ ID NO: 52 - protein, 6 aa, Artificial Sequence
  Description of Artificial Sequence: Synthetic peptide
DGTVLK

SEQ ID NO: 53 - protein, 6 aa, Artificial Sequence
  Description of Artificial Sequence: Synthetic peptide
EGLIVK

SEQ ID NO: 54 - protein, 6 aa, Artificial Sequence
  Description of Artificial Sequence: Synthetic peptide
EGVMIR

SEQ ID NO: 55 - protein, 6 aa, Artificial Sequence
  Description of Artificial Sequence: Synthetic peptide
EGLMVK

SEQ ID NO: 56 - protein, 6 aa, Artificial Sequence
  Description of Artificial Sequence: Synthetic peptide
EGVMVK

SEQ ID NO: 57 - protein, 6 aa, Artificial Sequence
  Description of Artificial Sequence: Synthetic peptide
EGLMAK

SEQ ID NO: 58 - protein, 6 aa, Artificial Sequence
  Description of Artificial Sequence: Synthetic peptide
EGVIAK

SEQ ID NO: 59 - protein, 6 aa, Artificial Sequence
  Description of Artificial Sequence: Synthetic peptide
EGYVLK

SEQ ID NO: 60 - protein, 6 aa, Artificial Sequence
  Description of Artificial Sequence: Synthetic peptide
EGVVIR

SEQ ID NO: 61 - protein, 6 aa, Artificial Sequence
  Description of Artificial Sequence: Synthetic peptide
EGYVAV

SEQ ID NO: 62 - protein, 6 aa, Artificial Sequence
  Description of Artificial Sequence: Synthetic peptide
EGIIMK

SEQ ID NO: 63 - protein, 5 aa, Artificial Sequence
  Description of Artificial Sequence: Synthetic peptide
AVAFK

SEQ ID NO: 64 - protein, 5 aa, Artificial Sequence
  Description of Artificial Sequence: Synthetic peptide
AIAYK

SEQ ID NO: 65 - protein, 5 aa, Artificial Sequence
  Description of Artificial Sequence: Synthetic peptide
ALAYK

SEQ ID NO: 66 - protein, 5 aa, Artificial Sequence
  Description of Artificial Sequence: Synthetic peptide
AIAYK

SEQ ID NO: 67 - protein, 5 aa, Artificial Sequence
  Description of Artificial Sequence: Synthetic peptide
WWKMK

SEQ ID NO: 68 - protein, 5 aa, Artificial Sequence
  Description of Artificial Sequence: Synthetic peptide
LLKMK

SEQ ID NO: 69 - protein, 5 aa, Artificial Sequence
  Description of Artificial Sequence: Synthetic peptide
WLKLK

SEQ ID NO: 70 - protein, 5 aa, Artificial Sequence
  Description of Artificial Sequence: Synthetic peptide
WIKLK

SEQ ID NO: 71 - protein, 5 aa, Artificial Sequence
  Description of Artificial Sequence: Synthetic peptide
WLKIK

SEQ ID NO: 72 - protein, 5 aa, Artificial Sequence
  Description of Artificial Sequence: Synthetic peptide
WVKDK

SEQ ID NO: 73 - protein, 5 aa, Artificial Sequence
  Description of Artificial Sequence: Synthetic peptide
AIKCK

SEQ ID NO: 74 - protein, 5 aa, Artificial Sequence
  Description of Artificial Sequence: Synthetic peptide
IIKLR

SEQ ID NO: 75 - protein, 5 aa, Artificial Sequence
  Description of Artificial Sequence: Synthetic peptide
HFKIK

SEQ ID NO: 76 - protein, 5 aa, Artificial Sequence
  Description of Artificial Sequence: Synthetic peptide
IVKYV

SEQ ID NO: 77 - protein, 298 aa, Paramecium bursaria Chlorella virus 1
MAITKPLLAATLENIEDVQFPCLATPKIDGIRSVKQTQMLSRTFKPIRNSVMNRLLTELLPEGSDGEISIEGATFQDTTSAVMTGHKMYNAKFSYYWFDYVTDDPLKKYIDRVEDMKNYITVHPHILEHAQVKIIPLIPVEINNITELLQYERDVLSKGFEGVMIRKPDGKYKFGRSTLKEGILLKMKQFKDAEATIISMTALFKNTNTKTKDNFGYSKRSTHKSGKVEEDVMGSIEVDYDGVVFSIGTGFDADQRRDFWQNKESYIGKMVKFKYFEMGSKDCPRFPVFIGIRHEEDR

SEQ ID NO: 78 - protein, 306 aa, Burkholderia pseudomallei
MSGVPYGFKPNLAATLTKPELIKFPVWASPKIDGIRCVFFGGVAYSRSLKPIPNPVVQEFAKAYANLLEGLDGELTVGSPTDANCMQNSMAVMSKAAAPDFTFHVFDWFHPAQAHIEFWQRSDVVEDRIVQFYDRYPEVDIRAAPQVLCTSLAHLDTNEARWLADGYEGMMIRDHCGRYKFGRSTEREGGLVKVKRFTDAEAIVIGFEEEMHNANEAKRDATGRTERSTSKAGLHGKGTLGALVVKNERGIVFNIGTGFTAAQRADYWANHPSLFGKMVKFKHFDHGTVDAPRHPVFIGFRHPEDM

SEQ ID NO: 79 - protein, 268 aa, Haemophilus influenza
MKFYRTLLLFFASSFAFANSDLMLLHTYNNQPIEGWVMSEKLDGVRGYWNGKQLLTRQGQRLSPPAYFIKDFPPFAIDGELFSERNHFEEISTITKSFKGDGWEKLKLYVFDVPDAEGNLFERLAKLKAHLLEHPTTYIEIIEQIPVKDKTHLYQFLAQVENLQGEGVVVRNPNAPYERKRSSQILKLKTARGEECTVIAHHKGKGQFENVMGALTCKNHRGEFKIGSGFNLNERENPPPIGSVITYKYRGITNSGKPRFATYWREKK

SEQ ID NO: 80 - protein, 268 aa, Haemophilus influenza
MKFYRTLLLFFASSFAFANSDLMLLHTYNNQPIEGWVMSEKLDGVRGYWNGKQLLTRQGQRLSPPAYFIKDFPPFAIDGELFSERNHFEEISSITKSFKGDGWEKLKLYVFDVPDAEGNLFERLAKLKAHLLEHPTTYIEIIEQIPVKDKTHLYQFLAQVENLQGEGVVVRNPNAPYERKRSSQILKLKTARGEECTVIAHHKGKGQFENVMGALTCKNHRGEFKIGSGFNLNERENPPPIGSVITYKYRGITNSGKPRFATYWREKK

SEQ ID NO: 81 - protein, 268 aa, Haemophilus influenza
MKFYRTLLLFFASSFAFANSDLMLLHTYNNQPIEGWVMSEKLDGVRGYWNGKQLLTRQGQRLSPPAYFIKDFPPFAIDGELFSERNHFEEISSITKSFKGDGWEKLKLYVFDVPDAEGNLFERLAKLKAHLLEHPTTYIEIIEQIPVKDKTHLYQFLAQVENLQGEGVVVRNPNAPYERKRSSQILKLKTARDEECTVIAHHKGKGQFENVMGALTCKNHRGEFKIGSGFNLNERENPPPIGSVITYKYRGITNSGKPRFATYWREKK

SEQ ID NO: 82 - protein, 246 aa, Haemophilus influenza
MLLHTYNNQPIEGWVMSEKLDGVRGYWNGKQLLTRQGQRLSPPAYFIKDFPPFAIDGELFSERNHFEEISSITKSFKGDGWEKLKLYVFDVPDAEGNLFERLAKLKAHLLEHPTTYIEIIEQIPVKDKTHLYQFLAQVENLQGEGVVVRNPNAPYERKRSSQILKLKTARDEECTVIAHHKGKGQFENVMGALTCKNHRGEFKIGSGFNLNERENPPPIGSVITYKYRGITNSGKPRFATYWREKK

SEQ ID NO: 83 - DNA, 12 bp, Artificial Sequence
  Description of Artificial Sequence: Synthetic oligonucleotide
aaaaaaaaaaaa

SEQ ID NO: 84 - protein, 6 aa, Artificial Sequence
  Description of Artificial Sequence: Synthetic peptide
  MOD_RES (2)..(2): Any amino acid
  MOD_RES (5)..(5): Any amino acid
KXDGXR